European Patent Application EP 4 183 417 A1, published May 24, 2023. Title: AN IMMUNOTHERAPEUTIC FOR PROSTATE CANCER TREATMENT. Applicant: Hexamer Therapeutics, Inc. Application EP. The sequence listing filed with the application follows.

SEQUENCE LISTING (78 sequences)

SEQ ID NO: 1-2 - skipped (2 entries)

SEQ ID NO: 3 - protein, 7 aa, synthetic construct
  REGION 1..7: note = Synthetic peptide
LRSIGKD

SEQ ID NO: 4 - protein, 7 aa, synthetic construct
  REGION 1..7: note = Synthetic peptide
LRSIGRD

SEQ ID NO: 5 - protein, 7 aa, synthetic construct
  REGION 1..7: note = Synthetic peptide
IREISRA

SEQ ID NO: 6 - protein, 7 aa, synthetic construct
  REGION 1..7: note = Synthetic peptide
IREVAQS

SEQ ID NO: 7 - protein, 7 aa, synthetic construct
  REGION 1..7: note = Synthetic peptide
IRDIAKA

SEQ ID NO: 8 - protein, 7 aa, synthetic construct
  REGION 1..7: note = Synthetic peptide
IRDIGRA

SEQ ID NO: 9 - protein, 7 aa, synthetic construct
  REGION 1..7: note = Synthetic peptide
IRDVGQS

SEQ ID NO: 10 - protein, 7 aa, synthetic construct
  REGION 1..7: note = Synthetic peptide
IRDLAKG

SEQ ID NO: 11 - protein, 7 aa, synthetic construct
  REGION 1..7: note = Synthetic peptide
VKDVARG

SEQ ID NO: 12 - protein, 7 aa, synthetic construct
  REGION 1..7: note = Synthetic peptide
IRDIGNS

SEQ ID NO: 13 - protein, 7 aa, synthetic construct
  REGION 1..7: note = Synthetic peptide
IKDLARG

SEQ ID NO: 14 - protein, 7 aa, synthetic construct
  REGION 1..7: note = Synthetic peptide
IKKLKKK

SEQ ID NO: 15 - protein, 7 aa, synthetic construct
  REGION 1..7: note = Synthetic peptide
IRSIGKE

SEQ ID NO: 16 - protein, 7 aa, synthetic construct
  REGION 1..7: note = Synthetic peptide
IRSIGRE

SEQ ID NO: 17 - protein, 7 aa, synthetic construct
  REGION 1..7: note = Synthetic peptide
IKSIGRE

SEQ ID NO: 18 - protein, 7 aa, synthetic construct
  REGION 1..7: note = Synthetic peptide
IRSIGRG

SEQ ID NO: 19 - protein, 28 aa, synthetic construct
  REGION 1..28: note = Synthetic peptide
LRSIGKDLRSIGKDLRSIGKDLRSIGKD

SEQ ID NO: 20 - protein, 29 aa, synthetic construct
  REGION 1..29: note = Synthetic peptide
LRSIGKDLRSIGKDLRSIGKDLRSIGKDS

SEQ ID NO: 21 - protein, 28 aa, synthetic construct
  REGION 1..28: note = Synthetic peptide
LRSIGKDLRSIGRDLRSIGKDLRSIGRD

SEQ ID NO: 22 - protein, 28 aa, synthetic construct
  REGION 1..28: note = Synthetic peptide
IREISRAIREVAQSIRDIAKAIREIGKS

SEQ ID NO: 23 - protein, 28 aa, synthetic construct
  REGION 1..28: note = Synthetic peptide
IRDIGRAIRDVGQSIRDLAKGIRDISKG

SEQ ID NO: 24 - protein, 28 aa, synthetic construct
  REGION 1..28: note = Synthetic peptide
VKDVARGIRDIGNSIKDLARGIRDIGRG

SEQ ID NO: 25 - protein, 28 aa, synthetic construct
  REGION 1..28: note = monomeric hC peptides
IRSIGKEIRSIGREIKSIGREIRSIGRG

SEQ ID NO: 26 - protein, 28 aa, synthetic construct
  REGION 1..28: note = monomeric hC peptides
IRSIGKEIRSIGREIRSIGKEIRSIGRE

SEQ ID NO: 27 - protein, 28 aa, synthetic construct
  REGION 1..28: note = monomeric hC peptides
IRSIGKEIRSIGREIRSIGREIRSIGRE

SEQ ID NO: 28 - protein, 10 aa, synthetic construct
  REGION 1..10: note = GnRH peptide sequence pattern
  SITE 1: note = MISC_FEATURE - Xaa ia a polar or charged amino acid
  SITE 5: note = MISC_FEATURE - Xaa ia a polar amino acid
  SITE 7: note = MISC_FEATURE - Xaa ia a hydrophobic or amphipathic amino acid
  SITE 8: note = MISC_FEATURE - Xaa ia a hydrophobic, amphipathic, charged, or polar amino acid
XHWSXGXXPG

SEQ ID NO: 29 - protein, 10 aa, synthetic construct
  REGION 1..10: note = GnRH peptide
QHWSYGLRPG

SEQ ID NO: 30 - protein, 10 aa, synthetic construct
  REGION 1..10: note = GnRH peptide
QHWSHGWLPG

SEQ ID NO: 31 - protein, 10 aa, synthetic construct
  REGION 1..10: note = GnRH peptide
EHWSYGLRPG

SEQ ID NO: 32 - protein, 10 aa, synthetic construct
  REGION 1..10: note = GnRH peptide
QHWSYGWYPG

SEQ ID NO: 33 - protein, 10 aa, synthetic construct
  REGION 1..10: note = GnRH peptide
EHWSYGLQPG

SEQ ID NO: 34 - protein, 10 aa, synthetic construct
  REGION 1..10: note = GnRH peptide
QHWSHGWYPG

SEQ ID NO: 35 - protein, 11 aa, synthetic construct
  REGION 1..11: note = Synthesized
  SITE 1: note = MISC_FEATURE - Xaa is Gly or Val
XQHWSYGLRPG

SEQ ID NO: 36 - protein, 4 aa, synthetic construct
  REGION 1..4: note = Synthetic peptide
GEDC

SEQ ID NO: 37 - protein, 5 aa, synthetic construct
  REGION 1..5: note = residues of GnRH peptides
DGEGC

SEQ ID NO: 38 - protein, 15 aa, Clostridium botulinum
LLVLVFTFSLIISAS

SEQ ID NO: 39 - protein, 15 aa, Clostridium botulinum
FSLIISASSANQVYA

SEQ ID NO: 40 - protein, 15 aa, Clostridium perfringens
RLITAMILAGAISIG

SEQ ID NO: 41 - protein, 15 aa, Staphylococcus aureus
NRNFLQRIWDAIVAF

SEQ ID NO: 42 - protein, 15 aa, synthetic construct
  REGION 1..15: note = Mycobacterium
TPSTDSTAFTAVAQE

SEQ ID NO: 43 - protein, 15 aa, synthetic construct
  REGION 1..15: note = Mycobacterium
RGQFDRFTRDTGIAV

SEQ ID NO: 44 - protein, 15 aa, synthetic construct
  REGION 1..15: note = Mycobacterium
GQFDRFTRDTGIAVN

SEQ ID NO: 45 - protein, 15 aa, synthetic construct
  REGION 1..15: note = Mycobacterium
FTRDTGIAVNLVEAG

SEQ ID NO: 46 - protein, 15 aa, synthetic construct
  REGION 1..15: note = Mycobacterium
VIGLAAVTIAAAATA

SEQ ID NO: 47 - protein, 15 aa, Clostridium tetani
IEIIDSLQWDRNLRI

SEQ ID NO: 48 - protein, 15 aa, Clostridium tetani
EIIDSLQWDRNLRIN

SEQ ID NO: 49 - protein, 15 aa, Clostridium tetani
IIDSLQWDRNLRINL

SEQ ID NO: 50 - protein, 15 aa, Mycobacterium tuberculosis
EISTNIRQAGVQYSR

SEQ ID NO: 51 - protein, 20 aa, Mycobacterium tuberculosis
SEFAYGSFVRTVSLPVGADE

SEQ ID NO: 52 - protein, 15 aa, Mumps virus
GTYRLIPNARANLTA

SEQ ID NO: 53 - protein, 16 aa, Plasmodium falciparum
EENVEENVEENVEENV

SEQ ID NO: 54 - protein, 20 aa, Human immunodeficiency virus type 1
AFSPEVIPMFSALSEGATPQ

SEQ ID NO: 55 - protein, 21 aa, Hepatitis C virus
GEGAVQWMNRLIAFASRGNHV

SEQ ID NO: 56 - protein, 11 aa, Influenza A virus
FVFTLTVPSER

SEQ ID NO: 57 - protein, 20 aa, Influenza A virus
LVVPRYAFAMERNAGSGIII

SEQ ID NO: 58 - protein, 7 aa, synthetic construct
  REGION 1..7: note = TLR-4 agonist
APPHALS

SEQ ID NO: 59 - protein, 19 aa, synthetic construct
  REGION 1..19: note = TCE1
LTAELKIYSVIQAEINKHL

SEQ ID NO: 60 - protein, 23 aa, synthetic construct
  REGION 1..23: note = TCE2
FNNFTVSFWLRVPRVSASHLEQY

SEQ ID NO: 61 - protein, 14 aa, synthetic construct
  REGION 1..14: note = TCE3
GQEAFSHIRIPLPH

SEQ ID NO: 62 - protein, 15 aa, synthetic construct
  REGION 1..15: note = TCE4
FQDAYNAAGGHNAVF

SEQ ID NO: 63 - protein, 4 aa, synthetic construct
  REGION 1..4: note = Synthesized
GPGP

SEQ ID NO: 64 - protein, 5 aa, synthetic construct
  REGION 1..5: note = Synthesized
GPGPG

SEQ ID NO: 65 - protein, 6 aa, synthetic construct
  REGION 1..6: note = Synthesized
GPGPGC

SEQ ID NO: 66 - protein, 6 aa, synthetic construct
  REGION 1..6: note = Synthesized
SGPGPG

SEQ ID NO: 67 - protein, 67 aa, synthetic construct
  REGION 1..67: note = GnRH_Hex_TCE2
GQHWSYGLRPGGDIRSIGKEIRSIGREIKSIGREIRSIGRGPGPFNNFTVSFWLRVPRVSASHLEQY

SEQ ID NO: 68 - protein, 58 aa, synthetic construct
  REGION 1..58: note = TCE3_Hex_TCE4
GQEAFSHIRIPLPHDIRSIGKEIRSIGREIRSIGKEIRSIGREFQDAYNAAGGHNAVF

SEQ ID NO: 69 - protein, 56 aa, synthetic construct
  REGION 1..56: note = GnRH_Hex_GnRH
GQHWSYGLRPGGSGDIRSIGKEIRSIGREIRSIGREIRSIGREGSGQHWSYGLRPG

SEQ ID NO: 70 - protein, 15 aa, synthetic construct
  REGION 1..15: note = GnRH
QHWSYGLRPGDGEGC

SEQ ID NO: 71 - protein, 57 aa, synthetic construct
  REGION 1..57: note = GnRH_TCE1
QHWSYGLRPGSGPGPGLTAELKIYSVIQAEINKHLGPGPGSFERFEIFPKEGPGPGC

SEQ ID NO: 72 - protein, 14 aa, synthetic construct
  REGION 1..14: note = GnRH peptide with synthetic peptide
QHWSYGLRPGGEDC

SEQ ID NO: 73 - protein, 14 aa, synthetic construct
  REGION 1..14: note = GnRH peptide with synthetic peptide
QHWSHGWLPGGEDC

SEQ ID NO: 74 - protein, 14 aa, synthetic construct
  REGION 1..14: note = GnRH peptide with synthetic peptide
EHWSYGLRPGGEDC

SEQ ID NO: 75 - protein, 14 aa, synthetic construct
  REGION 1..14: note = GnRH peptide with synthetic peptide
QHWSYGWYPGGEDC

SEQ ID NO: 76 - protein, 14 aa, synthetic construct
  REGION 1..14: note = GnRH peptide with synthetic peptide
EHWSYGLQPGGEDC

SEQ ID NO: 77 - protein, 14 aa, synthetic construct
  REGION 1..14: note = GnRH peptide with synthetic peptide
QHWSHGWYPGGEDC

SEQ ID NO: 78 - protein, 11 aa, synthetic construct
  REGION 1..11: note = TCE1
SFERFEIFPKE